European Patent Specification EP 4 204 591 B1, published December 25, 2024. Title: Method of assessing the circadian rhythm of a subject having cancer and/or assessing a timing of administration of a medicament to said subject having cancer. Applicant: Moreira Borralho Relógio, Angela. The sequence listing filed with the application follows.

SEQUENCE LISTING (19 sequences)

SEQ ID NO: 1 - DNA, 1878 bp, Human
atggcagaccagagaatggacatttcttcaaccatcagtgatttcatgtccccgggccccaccgacctgctttccagctctcttggtaccagtggtgtggattgcaaccgcaaacggaaaggcagctccactgactaccaagaaagcatggacacagacaaagatgaccctcatggaaggttagaatatacagaacaccaaggaaggataaaaaatgcaagggaagctcacagtcagattgaaaagcggcgtcgggataaaatgaacagttttatagatgaattggcttctttggtaccaacatgcaacgcaatgtccaggaaattagataaacttactgtgctaaggatggctgttcagcacatgaaaacattaagaggtgccaccaatccatacacagaagcaaactacaaaccaacttttctatcagacgatgaattgaaacacctcattctcagggcagcagatggatttttgtttgtcgtaggatgtgaccgagggaagatactctttgtctcagagtctgtcttcaagatcctcaactacagccagaatgatctgattggtcagagtttgtttgactacctgcatcctaaagatattgccaaagtcaaggagcagctctcctcctctgacaccgcaccccgggagcggctcatagatgcaaaaactggacttccagttaaaacagatataacccctgggccatctcgattatgttctggagcacgacgttctttcttctgtaggatgaagtgtaacaggccttcagtaaaggttgaagacaaggacttcccctctacctgctcaaagaaaaaagatcgaaaaagcttctgcacaatccacagcacaggctatttgaaaagctggccacccacaaagatggggctggatgaagacaacgaaccagacaatgaggggtgtaacctcagctgcctcgtcgcaattggacgactgcattctcatgtagttccacaaccagtgaacggggaaatcagggtgaaatctatggaatatgtttctcggcacgcgatagatggaaagtttgtttttgtagaccagagggcaacagctattttggcatatttaccacaagaacttctaggcacatcgtgttatgaatattttcaccaagatgacataggacatcttgcagaatgtcataggcaagttttacagacgagagaaaaaattacaactaattgctataaatttaaaatcaaagatggttcttttatcacactacggagtcgatggttcagtttcatgaacccttggaccaaggaagtagaatatattgtctcaactaacactgttgttttagccaacgtcctggaaggcggggacccaaccttcccacagctcacagcatccccccacagcatggacagcatgctgccctctggagaaggtggcccaaagaggacccaccccactgttccagggattccagggggaacccgggctggggcaggaaaaataggccgaatgattgctgaggaaatcatggaaatccacaggataagagggtcatcgccttctagctgtggctccagcccattgaacatcacgagtacgcctccccctgatgcctcttctccaggaggcaagaagattttaaatggagggactccagacattccttccagtggcctactatcaggccaggctcaggagaacccaggttatccatattctgatagttcttctattcttggtgagaacccccacataggtatagacatgattgacaacgaccaaggatcaagtagtcccagtaatgatgaggcagcaatggctgtcatcatgagcctcttggaagcagatgctggactgggtggccctgttgactttagtgacttgccatggccgctgtaa

SEQ ID NO: 2 - DNA, 1911 bp, Human
atggcggcggaagaggaggctgcggcgggaggtaaagtgttgagagaggagaaccagtgcattgctcctgtggtttccagccgcgtgagtccagggacaagaccaacagctatggggtctttcagctcacacatgacagagtttccacgaaaacgcaaaggaagtgattcagacccatcccagtcaggaatcatgacagaaaaagtggtggaaaagctttctcagaatccccttacctatcttctttcaacaaggatagaaatatcagcctccagtggcagcagagtggaagatggtgaacaccaagttaaaatgaaggccttcagagaagctcatagccaaactgaaaagcggaggagagataaaatgaataacctgattgaagaactgtctgcaatgatccctcagtgcaaccccatggcgcgtaaactggacaaacttacagttttaagaatggctgttcaacacttgagatctttaaaaggcttgacaaattcttatgtgggaagtaattatagaccatcatttcttcaggataatgagctcagacatttaatccttaagactgcagaaggcttcttatttgtggttggatgtgaaagaggaaaaattctcttcgtttctaagtcagtctccaaaatacttaattatgatcaggctagtttgactggacaaagcttatttgacttcttacatccaaaagatgttgccaaagtaaaggaacaactttcttcttttgatatttcaccaagagaaaagctaatagatgccaaaactggtttgcaagttcacagtaatctccacgctggaaggacacgtgtgtattctggctcaagacgatcttttttctgtcggataaagagttgtaaaatctctgtcaaagaagagcatggatgcttacccaactcaaagaagaaagagcacagaaaattctatactatccattgcactggttacttgagaagctggcctccaaatattgttggaatggaagaagaaaggaacagtaagaaagacaacagtaattttacctgccttgtggccattggaagattacagccatatattgttccacagaacagtggagagattaatgtgaaaccaactgaatttataacccggtttgcagtgaatggaaaatttgtctatgtagatcaaagggcaacagcgattttaggatatctgcctcaggaacttttgggaacttcttgttatgaatattttcatcaagatgaccacaataatttgactgacaagcacaaagcagttctacagagtaaggagaaaatacttacagattcctacaaattcagagcaaaagatggctcttttgtaactttaaaaagccaatggtttagtttcacaaatccttggacaaaagaactggaatatattgtatctgtcaacactttagttttgggacatagtgagcctggagaagcatcatttttaccttgtagctctcaatcatcagaagaatcctctagacagtcctgtatgagtgtacctggaatgtctactggaacagtacttggtgctggtagtattggaacagatattgcaaatgaaattctggatttacagaggttacagtcttcttcataccttgatgattcgagtccaacaggtttaatgaaagatactcatactgtaaactgcaggagtatgtcaaataaggagttgtttccaccaagtccttctgaaatgggggagctagaggctaccaggcaaaaccagagtactgttgctgtccacagccatgagccactcctcagtgatggtgcacagttggatttcgatgccctatgtgacaatgatgacacagccatggctgcatttatgaattacttagaagcagaggggggcctgggagaccctggggacttcagtgacatccagtggaccctctag

SEQ ID NO: 3 - DNA, 3873 bp, Human
atgagtggccccctagaaggggctgatgggggaggggaccccaggcctggggaatcattttgtcctgggggcgtcccatcccctgggcccccacagcaccggccttgcccaggccccagcctggccgatgacaccgatgccaacagcaatggttcaagtggcaatgagtccaacgggcatgagtctagaggcgcatctcagcggagctcacacagctcctcctcaggcaacggcaaggactcagccctgctggagaccactgagagcagcaagagcacaaactctcagagcccatccccacccagcagttccattgcctacagcctcctgagtgccagctcagagcaggacaacccgtccaccagtggctgcagcagtgaacagtcagcccgggcaaggactcagaaggaactcatgacagcacttcgagagctcaagcttcgactgccgccagagcgccggggcaagggccgctctgggaccctggccacgctgcagtacgcactggcctgtgtcaagcaggtgcaggccaaccaggaatactaccagcagtggagcctggaggagggcgagccttgctccatggacatgtccacctataccctggaggagctggagcacatcacgtctgagtacacacttcagaaccaggataccttctcagtggctgtctccttcctgacgggccgaatcgtctacatttcggagcaggcagccgtcctgctgcgttgcaagcgggacgtgttccggggtacccgcttctctgagctcctggctccccaggatgtgggagtcttctatggttccactgctccatctcgcctgcccacctggggcacaggggcctcagcaggttcaggcctcagggactttacccaggagaagtccgtcttctgccgtatcagaggaggtcctgaccgggatccagggcctcggtaccagccattccgcctaaccccgtatgtgaccaagatccgggtctcagatggggcccctgcacagccgtgctgcctgctgattgcagagcgcatccattcgggttacgaagctccccggataccccctgacaagaggattttcactacgcggcacacacccagctgcctcttccaggatgtggatgaaagggctgcccccctgctgggctacctgccccaggacctcctgggggccccagtgctcctgttcctgcatcctgaggaccgacccctcatgctggctatccacaagaagattctgcagttggcgggccagccctttgaccactcccctatccgcttctgtgcccgcaacggggagtatgtcaccatggacaccagctgggctggctttgtgcacccctggagccgcaaggtagccttcgtgttgggccgccacaaagtacgcacggcccccctgaatgaggacgtgttcactcccccggcccccagcccagctccctccctggacactgatatccaggagctgtcagagcagatccaccggctgctgctgcagcccgtccacagccccagccccacgggactctgtggagtcggcgccgtgacatccccaggccctctccacagccctgggtcctccagtgatagcaacgggggtgatgcagaggggcctgggcctcctgcgccagtgactttccagcagatctgtaaggatgtgcatctggtgaagcaccagggccagcagctttttattgagtctcgggcccggcctcagtcccggccccgcctccctgctacaggcacgttcaaggccaaggcccttccctgccaatccccagacccagagctggaggcgggttctgctcccgtccaggccccactagccttggtccctgaggaggccgagaggaaagaagcctccagctgctcctaccagcagatcaactgcctggacagcatcctcaggtacctggagagctgcaacctccccagcaccactaagcgtaaatgtgcctcctcctcctcctataccacctcctcagcctctgacgacgacaggcagaggacaggtccagtctctgtggggaccaagaaagatccgccgtcagcagcgctgtctggggagggggccaccccacggaaggagccagtggtgggaggcaccctgagcccgctcgccctggccaataaggcggagagtgtggtgtccgtcaccagtcagtgtagcttcagctccaccatcgtccatgtgggagacaagaagcccccggagtcggacatcatcatgatggaggacctgcctggcctagccccaggcccagcccccagcccagcccccagccccacagtagcccctgacccagccccagacgcctaccgtccagtggggctgaccaaggccgtgctgtccctgcacacacagaaggaagagcaagccttcctcagccgcttccgagacctgggcaggctgcgtggactcgacagctcttccacagctccctcagcccttggcgagcgaggctgccaccacggccccgcacccccaagccgccgacaccactgccgatccaaagccaagcgctcacgccaccaccagaaccctcgggctgaagcgccctgctatgtctcacacccctcacccgtgccaccctccaccccctggcccaccccaccagccactacccccttcccagcggttgtccagccctaccctctcccagtgttctctcctcgaggaggcccccagcctcttccccctgctcccacatctgtgcccccagctgctttccccgcccctttggtgaccccaatggtggccttggtgctccctaactatctgttcccaaccccatccagctatccttatggggcactccagacccctgctgaagggcctcccactcctgcctcgcactccccttctccatccttgcccgccctcgccccgagtcctcctcaccgcccggactctccactgttcaactcgagatgcagctctccactccagctcaatctgctgcagctggaggagctcccccgtgctgagggggctgctgttgcaggaggccctgggagcagtgccgggcccccacctcccagtgcggaggctgctgagccagaggccagactggcggaggtcactgagtcctccaatcaggacgcactttccggctccagtgacctgctcgaacttctgctgcaagaggactcgcgctccggcacaggctccgcagcctcgggctccttgggctctggcttgggctctgggtctggttcaggctcccatgaagggggcagcacctcagccagcatcactcgcagcagccagagcagccacacaagcaaatactttggcagcatcgactcttccgaggctgaggctggggctgctcggggcggggctgagcctggggaccaggtgattaagtacgtgctccaggatcccatttggctgctcatggccaatgctgaccagcgcgtcatgatgacctaccaggtgccctccagggacatgacctctgtgctgaagcaggatcgggagcggctccgagccatgcagaagcagcagcctcggttttctgaggaccagcggcgggaactgggtgctgtgcactcctgggtccggaagggccaactgcctcgggctcttgatgtgatggcctgtgtggactgtgggagcagcacccaagatcctggtcaccctgatgacccactcttctcagagctggatggactggggctggagcccatggaagagggtggaggcgagcagggcagcagcggtggcggcagtggtgagggagagggctgcgaggaggcccaaggcggggccaaggcttcaagctctcaggacttggctatggaggaggaggaagaaggcaggagctcatccagtccagccttacctacagcaggaaactgcaccagctag

SEQ ID NO: 4 - DNA, 3768 bp, Human
atgaatggatacgcggaatttccgcccagccccagtaaccccaccaaggagcccgtggagccccagcccagccaggtcccactgcaggaagatgtggacatgagcagtggctccagtggacatgagaccaacgaaaactgctccacggggcgggactcgcagggcagtgactgtgacgacagtgggaaggagctggggatgctggtggagccaccggatgcccgccagagtccagatacctttagcctgatgatggcaaaatctgaacacaacccatctacaagtggctgcagtagcgaccagtcttcgaaagtggacacacacaaagaactgataaaaacactaaaggagctgaaggtccacctccctgcagacaagaaggccaagggcaaggccagtacgctggccaccttgaagtacgccctcaggagcgtgaagcaggtgaaagccaatgaagagtattaccagctgctgatgtccagcgagggtcacccctgtggagcagacgtgccctcctacaccgtggaggagatggagagcgttacctctgagcacattgtgaagaatgccgatatgtttgcggtggccgtgtccctggtgtctgggaagatcctgtacatctctgaccaggttgcatccatatttcactgtaaaagagatgccttcagcgatgccaagtttgtggagttcctggcgcctcacgatgtgggcgtgttccacagtttcacctccccgtacaagcttcccttgtggagcatgtgcagtggagcagattcttttactcaagaatgcatggaggagaaatctttcttttgccgtgtcagtgtccggaaaagccacgagaatgaaatccgctaccaccccttccgcatgacgccctacctggtcaaggtgcgggaccaacaaggtgctgagagtcagctttgctgccttctgctggcagagagagtgcactctggttatgaagcccctagaattcctcctgaaaagagaatttttacaaccacccatacaccaaattgtttgttccaggatgtggatgaaagggcggtccctctcctgggctacctacctcaggacctgattgaaaccccagtgctcgtgcagctccaccctagtgacaggcccttgatgctggccatccacaaaaagatcctgcagtcaggcgggcagcctttcgactattctcccattcggtttcgcgcccggaacggagagtacatcacgttggacaccagctggtccagcttcatcaacccatggagcaggaaaatctccttcatcattgggaggcacaaagtcagggtgggccctttgaatgaggacgtgtttgcagcccacccctgcacagaggagaaggccctgcaccccagcattcaggagctcacagagcagatccaccggctcctgctgcagcccgtcccccacagcggctccagtggctacgggagtctgggcagcaacgggtcccacgagcaccttatgagccagacctcctccagcgacagcaacggccatgaggactcacgccggaggagagccgaaatttgtaaaaatggtaacaagaccaaaaatagaagtcattattctcatgaatctggagaacaaaagaaaaaatccgttacagaaatgcaaactaatcccccagctgagaagaaagctgtccctgccatggaaaaggacagcctgggggtcagcttccccgaggagttggcctgcaagaaccagcccacctgctcctaccagcagatcagctgcttggacagcgtcatcaggtacttggagagctgcaatgaggctgccaccctgaagaggaaatgcgagttcccagcaaacgtcccagcgctaaggtccagtgataagcggaaggccacagtcagcccagggccacacgctggagaggcagagccgccctccagggtgaacagccgcacgggagtaggtacgcacctgacctcgctggcactgccgggcaaggcagagagtgtggcgtcgctcaccagccagtgcagctacagcagcaccatcgtccatgtgggagacaagaagccgcagccggagttagagatggtggaagatgctgcgagtgggccagaatccctggactgcctggcgggccctgccctggcctgtggtctcagccaagagaaggagcccttcaagaagctgggcctcaccaaggaggtactcgctgcacacacacagaaggaggagcagagcttcctgcagaagttcaaagaaataagaaaactcagcattttccagtcccactgccattactacttgcaagaaagatccaaggggcagccaagtgaacgaactgcccctggactaagaaatacttccggaatagattcaccttggaaaaaaacaggaaagaacagaaaattgaagtccaagcgggtcaaacctcgagactcatctgagagcaccggatctggggggcccgtgtccgcccggcccccgctggtgggcttgaacgccacagcctggtcaccctcagacacgtcccagtccagctgcccagccgtgccctttcccgccccagtgccagcagcttattcactgcccgtgtttccagcgccagggactgtggcagcacccccggcacctccccacgccagcttcacagtgcctgctgtgcccgtggacctccagcaccagtttgcagtccagcccccacctttccctgcccctttggcgcctgtcatggcattcatgctacccagttattccttcccctcggggaccccaaacctgccccaggccttcttccccagccagcctcagtttccgagccaccccacactcacatccgagatggcctctgcctcacagcctgagttccccagccggacctcgatccccagacagccatgtgcttgtccagccacccgggccaccccaccatcggccatgggtagggcctccccaccgctctttcagtcccgcagcagctcgcccctgcagctcaacctgctgcagctggaggaagcccctgagggtggcactggagccatggggaccacaggggccacagagacagcagctgtaggggcggactgcaaacctggcacttctcgggaccagcagccgaaggcgcctctgacccgtgatgaaccctcagacacacagaacagtgacgccctttccacgtcaagcggcctcctaaacctcctgctgaatgaggacctctgctcagcctcgggctctgctgcttcggagtctctgggctccggctcactgggctgcgacgcctccccgagtggggcaggcagtagtgacacaagtcataccagcaaatattttggaagcattgactcctcagagaataatcacaaagcaaaaatgaacactggtatggaagaaagtgagcatttcattaagtgcgtcctgcaggatcccatctggctgctgatggcagatgcggacagcagcgtcatgatgacgtaccagctgccttcccgaaatttagaagcggttttgaaggaggacagagagaagctgaagctcctacagaaactccagcccaggttcacggagagtcagaagcaggagctgcgcgaggtccaccagtggatgcagacgggcggcctgcccgcagccatcgacgtggcagaatgtgtttactgtgaaaacaaggaaaaaggtaatatttgcataccatatgaggaagatattccttctctgggactcagcgaagtgtcggacaccaaagaagacgaaaatggatcccccttgaatcacaggatcgaagagcagacgtaa

SEQ ID NO: 5 - DNA, 3633 bp, Human
atgccccgcggggaagctcctggccccgggagacggggggctaaggacgaggccctgggcgaagaatcgggggagcggtggagccccgagttccatctgcagaggaaattggcggacagcagccacagtgaacagcaagatcgaaacagagtttctgaagaacttatcatggttgtccaagaaatgaaaaaatacttcccctcggagagacgcaataaaccaagcactctagatgccctcaactatgctctccgctgtgtccacagcgttcaagcaaacagtgagtttttccagattctcagtcagaatggagcacctcaggcagatgtgagcatgtacagtcttgaggagctggccactatcgcttcagaacacacttccaaaaacacagatacctttgtggcagtattttcatttctgtctggaaggttagtgcacatttctgaacaggctgctttgatcctgaatcgtaagaaagatgtcctggcgtcttctcactttgttgacctgcttgcacctcaagacatgagggtattctacgcgcacactgccagagctcagcttcctttctggaacaactggacccaaagagcagctgcacggtatgaatgtgctccggtgaaaccttttttctgcaggatccgtggaggtgaagacagaaagcaagagaagtgtcactccccattccggatcatcccctatctgattcatgtacatcaccctgcccagccagaattggaatcggaaccttgctgtctcactgtggttgaaaagattcactctggttatgaagctcctcggatcccagtgaataaaagaatcttcaccaccacacacaccccagggtgtgtttttcttgaagtagatgaaaaagcagtgcctttgctgggttacctacctcaggacctgattggaacatcgatcctaagctacctgcaccctgaagatcgttctctgatggttgccatacaccaaaaagttttgaagtatgcagggcatcctccctttgaacattctcccattcgattttgtactcaaaacggagactacatcatactggattccagttggtccagctttgtgaatccctggagccggaagatttctttcatcattggtcggcataaagttcgaacgagcccactaaatgaggatgtttttgctaccaaaattaaaaagatgaacgataatgacaaagacataacagaattacaagaacaaatttacaaacttctcttacagccagttcacgtgagcgtgtccagcggctacgggagcctggggagcagcgggtcgcaggagcagcttgtcagcatcgcctcctccagtgaggccagtgggcaccgtgtggaggagacgaaggcggagcagatgaccttgcagcaggtctatgccagtgtgaacaaaattaaaaatctgggtcagcagctctacattgagtcaatgaccaaatcatcattcaagccagtgacggggacacgcacagaaccgaatggtggtggtgagtcagcgaatggtggtggtgaatgtaagacctttacttccttccaccaaacactgaaaaacaatagtgtgtacactgagccctgtgaggatttgaggaacgatgagcacagcccatcctatcaacagatcaactgtatcgacagtgtcatcagatacctgaagagctacaacattccagctttgaaaagaaagtgtatctcctgtacaaatacaacttcttcctcctcagaagaagacaaacagaaccacaaggcagatgatgtccaagccttacaagctggtttgcaaatcccagccatacctaaatcagaaatgccaacaaatggacggtccatagacacaggaggaggagctccacagatcctgtccacggcgatgctgagcttggggtcgggcataagccaatgcggttacagcagcaccattgtccatgtcccacccccagagacagccagggatgctaccctcttctgtgagccctggaccctgaacatgcagccagcccctttgacctcggaagaatttaaacacgtggggctcacagcggctgttctgtcagcgcacacccagaaggaagagcagaattatgttgataaattccgagaaaagatcctgtcatcaccctacagctcctatcttcagcaagaaagcaggagcaaagctaaatattcatattttcaaggagattctacttccaagcagacgcggtcggccggctgcaggaaagggaagcacaagcggaagaagctgccggagccgccagacagcagcagctcgaacaccggctctggtccccgcaggggagcgcatcagaacgcacagccctgctgcccctccgcggcctcctctccgcacacctcgagcccgaccttcccacctgccgccatggtgcccagccaggccccttacctcgtcccagcttttcccctcccagccgcgacctcacccggaagagaatacgcagcccccggaactgcaccggaaggcctgcatgggctgcccttgtccgagggcttgcagccttacccagctttcccttttccttacttggatacttttatgaccgttttcctgcctgacccccctgtctgtcctctgttgtcgccatcgtttttgccatgtccattcctgggggcgacagcctcttctgcgatatcaccctcaatgtcgtcagcaatgagtccaactctggacccacccccttcagtcaccagccaaaggagagaggaggaaaagtgggaggcacaaagcgaggggcacccgttcattacttcgagaagcagctcacccttgcagttaaacttacttcaggaagagatgcccagaccctctgaatctccagatcagatgagaaggaacacgtgcccacaaactgagtatcagtgtgttacaggcaacaatggcagtgagagcagtcctgctactaccggtgcactgtccacggggtcacctcccagggagaatccatcccatcctactgccagcgctctgtccacaggatcgcctcccatgaagaatccatcccatcctactgccagcgctctgtccacaggatcgcctcccatgaagaatccatcccatcctactgccagcacactgtccatgggattgcctcccagcaggactccatcccatcctactgccactgttctgtccacggggtcacctcccagcgaatccccatccagaactggttcagcagcatcaggaagcagcgacagcagtatataccttactagtagtgtttattcttctaaaatctcccaaaatgggcagcaatctcaggacgtacagaaaaaagaaacatttcctaatgtcgccgaagagcccatctggagaatgatacggcagacacctgagcgcattctcatgacataccaggtacctgagagggttaaagaagttgtactaaaagaagacctggaaaagctagaaagtatgaggcagcagcagccccagttttctcatgggcaaaaggaggagctggctaaggtgtataattggattcaaagccagactgtcactcaagaaatcgacattcaagcctgtgtcacttgtgaaaatgaagattcagctgatggtgcggccacatcctgtggtcaggttctggtagaagacagctgttga

SEQ ID NO: 6 - DNA, 2541 bp, Human
atgttgtttaccgtaagctgtagtaaaatgagctcgattgttgacagagatgacagtagtatttttgatgggttggtggaagaagatgacaaggacaaagcgaaaagagtatctagaaacaaatctgaaaagaaacgtagagatcaatttaatgttctcattaaagaactgggatccatgcttcctggtaatgctagaaagatggacaaatctactgttctgcagaaaagcattgattttttacgaaaacataaagaaatcactgcacagtcagatgctagtgaaattcgacaggactggaaacctacattccttagtaatgaagagtttacacaattaatgttagaggctcttgatggtttttttttagcaatcatgacagatggaagcataatatatgtgtctgagagtgtaacttcattacttgaacatttaccatctgatcttgtggatcaaagtatatttaattttatcccagaaggggaacattcagaggtttataaaatactctctactcatctgctggaaagtgattcattaaccccagaatatttaaaatcaaaaaatcagttagaattctgttgtcacatgctgcgaggaacaatagacccaaaggagccatctacctatgaatatgtaaaatttataggaaatttcaaatctttaaacagtgtatcctcttcagcacacaatggttttgaaggaactatacaacgcacacataggccatcttatgaagatagagtttgttttgtagctactgtcaggttagctacacctcagttcatcaaggaaatgtgcactgttgaagaacccaatgaagagtttacatctagacatagtttagaatggaagtttctgtttctagatcacagggcaccacccataatagggtatttgccatttgaagttctgggaacatcaggctatgattactatcatgtggatgacctagaaaatttggcaaaatgtcatgagcacttaatgcaatatgggaaaggcaaatcatgttattataggttcctgactaaggggcaacagtggatttggcttcagactcattattatatcacttaccatcagtggaattcaaggccagagtttattgtttgtactcacactgtagtaagttatgcagaagttagggctgaaagacgacgagaacttggcattgaagagtctcttcctgagacagctgctgacaaaagccaagattctgggtcagataatcgtataaacacagtcagtctcaaggaagcattggaaaggtttgatcacagcccaaccccttctgcctcttctcggagttcaagaaaatcatctcacacggccgtctcagacccttcctcaacaccaaccaagatcccgacggatacgagcactccacccaggcagcatttaccagctcatgagaagatggtgcaaagaaggtcatcatttagtagtcagtccataaattcccagtctgttggttcatcattaacacagccagtgatgtctcaagctacaaatttaccaattccacaaggcatgtcccagtttcagttttcagctcaattaggagccatgcaacatctgaaagaccaattggaacaacggacacgcatgatagaagcaaatattcatcggcaacaagaagaactaagaaaaattcaagaacaacttcagatggtccatggtcaggggctgcagatgtttttgcaacaatcaaatcctgggttgaattttggttccgttcaactttcttctggaaattcatctaatatccagcaacttgcacctataaatatgcaaggccaagttgttcctactaaccagattcaaagtggaatgaatactggacacattggcacaactcagcacatgatacaacaacagactttacagagtacatcaactcagagtcaacaaaatgtactgagtgggcacagtcagcaaacatctctacccagtcagacacagagcactcttacagccccactgtataacactatggtgatttctcagcctgcagccggaagcatggtccagattccatctagtatgccacaaaacagcacccagagtgctgcagtaactacattcactcaggacaggcagataagattttctcaaggtcaacaacttgtgaccaaattagtgactgctcctgtagcttgtggggcagtcatggtacctagtactatgcttatgggccaggtggtgactgcatatcctacttttgctacacaacagcaacagtcacagacattgtcagtaacgcagcagcagcagcagcagagctcccaggagcagcagctcacttcagttcagcaaccatctcaggctcagctgacccagccaccgcaacaatttttacagacttctaggttgctccatgggaatccctcaactcaactcattctctctgctgcatttcctctacaacagagcaccttccctcagtcacatcaccagcaacatcagtctcagcaacagcagcaactcagccggcacaggactgacagcttgcccgacccttccaaggttcaaccacagtag

SEQ ID NO: 7 - DNA, 2475 bp, Human
atggatgaagatgagaaagacagagccaagagagcttctcgaaacaagtctgagaagaagcgtcgggaccagttcaatgttctcatcaaagagctcagttccatgctccctggcaacacgcggaaaatggacaaaaccaccgtgttggaaaaggtcatcggatttttgcagaaacacaatgaagtctcagcgcaaacggaaatctgtgacattcagcaagactggaagccttcattcctcagtaatgaagaattcacccagctgatgttggaggcattagatggcttcattatcgcagtgacaacagacggcagcatcatctatgtctctgacagtatcacgcctctccttgggcatttaccgtcggatgtcatggatcagaatttgttaaatttcctcccagaacaagaacattcagaagtttataaaatcctttcttcccatatgcttgtgacggattccccctccccagaatacttaaaatctgacagcgatttagagttttattgccatcttctcagaggcagcttgaacccaaaggaatttccaacttatgaatacataaaatttgtaggaaattttcgctcttacaacaatgtgcctagcccctcctgtaatggttttgacaacaccctttcaagaccttgccgggtgccactaggaaaggaggtttgcttcattgccaccgttcgtctggcaacaccacaattcttaaaggaaatgtgcatagttgacgaacctttagaggaattcacttcaaggcatagcttggaatggaaatttttatttctggatcacagagcacctccaatcataggatacctgccttttgaagtgctgggaacctcaggctatgactactaccacattgatgacctggagctcctggccaggtgtcaccagcacctgatgcagtttggcaaagggaagtcgtgttgctaccggtttctgaccaaaggtcagcagtggatctggctgcagactcactactacatcacctaccatcagtggaactccaagcccgagttcatcgtgtgcacacactcggtggtcagttacgcagatgtccgggtggaaaggaggcaggagctggctctggaagacccgccatccgaggccctccactcctcagcactaaaggacaagggctcaagcctggaacctcggcagcactttaacacactcgacgtgggtgcctcgggccttaataccagtcattcgccatcggcgtcctcaagaagttcccacaaatcctcgcacacagccatgtcagaacccacctccactcccaccaagctgatggcagaggccagcaccccggctttgccaagatcagccaccctgccccaagagttacctgtccccgggctcagccaggcagccaccatgccggcccctctgccttccccatcgtcctgcgacctcacacagcagctcctgcctcagaccgttctgcagagcacgcccgctcccatggcacagttttcggcacagttcagcatgttccagaccatcaaagaccagctagagcagcggacgcggatcctgcaggccaatatccggtggcaacaggaagagctccacaagatccaggagcagctctgcctggtccaggactccaacgtccagatgttcctgcagcagccagctgtatccctgagcttcagcagcacccagcgacctgaggctcagcagcagctacagcaaaggtcagctgcagtgactcagccccagctcggggcgggcccccaacttccagggcagatctcctctgcccaggtcacaagccagcacctgctcagagaatcaagtgtgatatcaacccagggtccaaagccaatgagaagctcacagctaatgcagagcagcggccgctctggaagcagcctagtgtccccgttcagcagcgccacagctgcgctcccgccaagtctgaatctgaccacacctgcttccacctcccaggatgccagccagtgccagcccagcccagacttcagccatgatcggcagctcaggctgttgctgagccagcccatccagcccatgatgcccgggtcctgtgacgcaaggcagccctcggaagtcagcaggacgggacggcaagtcaagtacgcccagagccagaccgtgtttcaaaatccagacgcacaccccgccaacagcagcagcgccccgatgcccgtcctgctgatggggcaggcggtgctccaccccagcttccctgcctcccaaccatcgcccctgcagcctgcacaggcccggcagcagccaccgcagcactacctgcaggtacaggcaccaacctctttgcacagtgagcagcaggactcgctacttctctccacctactcacaacagccagggaccctgggctacccccaaccacccccagcacagccccagcccctacgtcctccccgaagggtcagcagtctgtctgagtcgtcaggcctccagcagccgccccgataa

SEQ ID NO: 8 - DNA, 1761 bp, Human
atgggggtgaacgccgtgcactggttccgaaaggggctccggctccacgacaaccccgccctgaaggagtgcattcagggcgccgacaccatccgctgcgtctacatcctggacccctggttcgccggctcctccaatgtgggcatcaacaggtggcgatttttgcttcagtgtcttgaggatcttgatgccaatctacgaaaattaaactcccgtctgtttgtgattcgtggacaaccagcagatgtgtttcccaggcttttcaaggaatggaacattactaaactttcaattgagtatgattctgagccctttggaaaggaacgagacgcagctattaagaaactggcaactgaagctggagtagaagtcattgtaagaatttcacatacattatatgacctagacaagatcatagaactcaatggtggacaaccgcctctaacttataaaagattccagactctcatcagcaaaatggaaccactagagataccagtagagacaattacttcagaagtgatagaaaagtgcacaactcctctgtctgatgaccatgatgagaaatatggagtcccttcactggaagagctaggttttgatacagatggcttatcctctgcagtgtggccaggtggagaaactgaagcacttactcgtttggaaaggcatttggaaagaaaagcttgggtggcaaattttgaaagacctcgaatgaatgcgaattctctgcttgcaagccctactggacttagtccttatctccgatttggttgtttgtcatgtcgactgttttacttcaaactaacagatctctacaaaaaggtaaagaagaacagttcccctcccctttccctttatgggcaactgttatggcgtgaatttttctatacagcagcaacaaataatccacgctttgataaaatggaaggaaaccctatctgtgttcagattccttgggataaaaatcctgaggctttagccaaatgggcggaaggccggacaggctttccatggattgatgccatcatgacacagcttcgtcaggagggttggattcatcatctagccaggcatgcagttgcttgcttcctgacacgaggggacctgtggattagttgggaagaaggaatgaaggtatttgaagaattattgcttgatgcagattggagcataaatgctggaagttggatgtggctgtcttgtagttccttttttcaacagttttttcactgctattgccctgttggttttggtaggagaacagatcccaatggagactatatcaggcgttatttgcctgtcctaagaggcttccctgcaaaatatatctatgatccctggaatgcaccagaaggtatccaaaaggtagccaaatgtttgataggagttaattatcctaaaccaatggtgaaccatgctgaggcaagccgtttgaatatcgaaaggatgaaacagatctatcagcagctttcacgatatagaggactaggtcttctggcatcagtaccttctaatcctaatgggaatggaggcttcatgggatattctgcagaaaatatcccaggttgtagcagcagtggaagttgctctcaagggagtggtattttacactatgctcatggcgacagtcagcaaactcacctgttgaagcaaggaagaagctccatgggcactggtctcagtggtgggaaacgtcctagtcaggaagaggacacacagagtattggtcctaaagtccagagacagagcactaattag

SEQ ID NO: 9 - DNA, 1845 bp, Human
atgggcggggtccacgtcgcctaccggggcggagcgggggtggctggagcagtctggacagtcatggcggcgactgtggcgacggcggcagctgtggccccggcgccagcgcccggcacggacagcgcctcttcggtgcactggttccgcaaagggctgcgactccacgacaacccggcgttgctggcggccgtgcgcggggcgcgctgcgtgcgctgcgtttacattctcgacccgtggttcgcggcctcctcctcagtcgggatcaaccgatggaggttcctacttcagtctctggaagatttggacacaagtttaaggaaactgaactcccgcctgtttgtagtccggggacagccagccgacgtgttcccaaggctgttcaaggaatggggagtgacccgcttgacctttgaatatgactctgaaccctttgggaaagaacgggatgcagccatcatgaagatggccaaggaggctggtgtggaagtagtgacggagaattctcataccctctatgacctggacaggatcattgagctgaatgggcagaagccaccccttacatacaagcgctttcaggccatcatcagccgcatggagctgcccaagaagccagtgggcttggtgaccagccagcagatggagagctgcagggccgagatccaggagaaccacgacgagacctacggcgtgccctccctggaggagctggggttccccactgaaggacttggtccagctgtctggcagggaggagagacagaagctctggcccgcctggataagcacttggaacggaaggcctgggttgccaactatgagagaccccgaatgaacgccaactccctcctggccagccccacaggcctcagcccctacctgcgctttggttgtctctcctgccgcctcttctactaccgcctgtgggacctgtataaaaaggtgaagcggaacagcacacctcccctctccctatttgggcaactcctatggcgagagttcttctacacggcagctaccaacaaccccaggtttgaccgcatggaggggaaccccatctgcatccagatcccctgggaccgcaatcctgaggccctggccaagtgggctgagggcaagacaggcttcccttggattgatgccatcatgacccaactgaggcaggagggctggatccaccacctggcccggcatgccgtggcctgcttcctgacccgcggggacctctgggtcagctgggagagcggggtccgggtatttgatgagctgctcctggatgcagatttcagcgtgaacgcaggcagctggatgtggctgtcctgcagtgctttcttccagcagttcttccactgctactgccctgtgggctttggccgtcgcacggaccccagtggggactacatcaggcgatacctgcccaaattgaaagcgttcccctctcgatacatctatgagccctggaatgccccagagtcaattcagaaggcagccaagtgcatcattggtgtggactacccacggcccatcgtcaaccatgccgagaccagccggcttaacattgaacgaatgaagcagatttaccagcagctttcgcgctaccggggactctgtctactggcatctgtcccttcctgtgtggaagacctcagtcaccctgtggcagagcccagctcgagccaggctggcagcatgagcagtgcaggcccaagaccactacccagtggcccagcatcccccaaacgcaagctggaagcagccgaggaaccacctggtgaagaactcagcaaacgggcccgggtggcagagttgccaaccccagagctgccgagcaaggatgcctga

SEQ ID NO: 10 - DNA, 1845 bp, Human
atgacgaccctggactccaacaacaacacaggtggcgtcatcacctacattggctccagtggctcctccccaagccgcaccagccctgaatccctctatagtgacaactccaatggcagcttccagtccctgacccaaggctgtcccacctacttcccaccatcccccactggctccctcacccaagacccggctcgctcctttgggagcattccacccagcctgagtgatgacggctccccttcttcctcatcttcctcgtcgtcatcctcctcctccttctataatgggagcccccctgggagtctacaagtggccatggaggacagcagccgagtgtcccccagcaagagcaccagcaacatcaccaagctgaatggcatggtgttactgtgtaaagtgtgtggggacgttgcctcgggcttccactacggtgtgcacgcctgcgagggctgcaagggctttttccgtcggagcatccagcagaacatccagtacaaaaggtgtctgaagaatgagaattgctccatcgtccgcatcaatcgcaaccgctgccagcaatgtcgcttcaagaagtgtctctctgtgggcatgtctcgagacgctgtgcgttttgggcgcatccccaaacgagagaagcagcggatgcttgctgagatgcagagtgccatgaacctggccaacaaccagttgagcagccagtgcccgctggagacttcacccacccagcaccccaccccaggccccatgggcccctcgccaccccctgctccggtcccctcacccctggtgggcttctcccagtttccacaacagctgacgcctcccagatccccaagccctgagcccacagtggaggatgtgatatcccaggtggcccgggcccatcgagagatcttcacctacgcccatgacaagctgggcagctcacctggcaacttcaatgccaaccatgcatcaggtagccctccagccaccaccccacatcgctgggaaaatcagggctgcccacctgcccccaatgacaacaacaccttggctgcccagcgtcataacgaggccctaaatggtctgcgccaggctccctcctcctaccctcccacctggcctcctggccctgcacaccacagctgccaccagtccaacagcaacgggcaccgtctatgccccacccacgtgtatgcagccccagaaggcaaggcacctgccaacagtccccggcagggcaactcaaagaatgttctgctggcatgtcctatgaacatgtacccgcatggacgcagtgggcgaacggtgcaggagatctgggaggatttctccatgagcttcacgcccgctgtgcgggaggtggtagagtttgccaaacacatcccgggcttccgtgacctttctcagcatgaccaagtcaccctgcttaaggctggcacctttgaggtgctgatggtgcgctttgcttcgttgttcaacgtgaaggaccagacagtgatgttcctaagccgcaccacctacagcctgcaggagcttggtgccatgggcatgggagacctgctcagtgccatgttcgacttcagcgagaagctcaactccctggcgcttaccgaggaggagctgggcctcttcaccgcggtggtgcttgtctctgcagaccgctcgggcatggagaattccgcttcggtggagcagctccaggagacgctgctgcgggctcttcgggctctggtgctgaagaaccggcccttggagacttcccgcttcaccaagctgctgctcaagctgccggacctgcggaccctgaacaacatgcattccgagaagctgctgtccttccgggtggacgcccagtga

SEQ ID NO: 11 - DNA, 1740 bp, Human
atggaggtgaatgcaggaggtgtgattgcctatatcagttcttccagctcagcctcaagccctgcctcttgtcacagtgagggttctgagaatagtttccagtcctcctcctcttctgttccatcttctccaaatagctctaattctgataccaatggtaatcccaagaatggtgatctcgccaatattgaaggcatcttgaagaatgatcgaatagattgttctatgaaaacaagcaaatcgagtgcacctgggatgacaaaaagtcatagtggtgtgacaaaatttagtggcatggttctactgtgtaaagtctgtggggatgtggcgtcaggattccactatggagttcatgcttgcgaaggctgtaagggtttctttcggagaagtattcaacaaaacatccagtacaagaagtgcctgaagaatgaaaactgttctataatgagaatgaataggaacagatgtcagcaatgtcgcttcaaaaagtgtctgtctgttggaatgtcaagagatgctgttcggtttggtcgtattcctaagcgtgaaaaacagaggatgctaattgaaatgcaaagtgcaatgaagaccatgatgaacagccagttcagtggtcacttgcaaaatgacacattagtagaacatcatgaacagacagccttgccagcccaggaacagctgcgacccaagccccaactggagcaagaaaacatcaaaagctcttctcctccatcttctgattttgcaaaggaagaagtgattggcatggtgaccagagctcacaaggatacctttatgtataatcaagagcagcaagaaaactcagctgagagcatgcagccccagagaggagaacggattcccaagaacatggagcaatataatttaaatcatgatcattgcggcaatgggcttagcagccattttccctgtagtgagagccagcagcatctcaatggacagttcaaagggaggaatataatgcattacccaaatggtcatgccatttgtattgcaaatggacattgtatgaacttctccaatgcttatactcaaagagtatgtgatagagttccgatagatggattttctcagaatgagaacaagaatagttacctgtgcaacactggaggaagaatgcatctggtttgtccaatgagtaagtctccatatgtggatcctcataaatcaggacatgaaatctgggaagaattttcgatgagcttcactccagcagtgaaagaagtggtggaatttgcaaagcgtattcctgggttcagagatctctctcagcatgaccaggtcaaccttttaaaggctgggacttttgaggttttaatggtacggttcgcatcattatttgatgcaaaggaacgtactgtcacctttttaagtggaaagaaatatagtgtggatgatttacactcaatgggagcaggggatctgctaaactctatgtttgaatttagtgagaagctaaatgccctccaacttagtgatgaagagatgagtttgtttacagctgttgtcctggtatctgcagatcgatctggaatagaaaacgtcaactctgtggaggctttgcaggaaactctcattcgtgcactaaggaccttaataatgaaaaaccatccaaatgaggcctctatttttacaaaactgcttctaaagttgccagatcttcgatctttaaacaacatgcactctgaggagctcttggcctttaaagttcacccttaa

SEQ ID NO: 12 - DNA, 1572 bp, Human
atggagtcagctccggcagcccccgaccccgccgccagcgagccaggcagcagcggcgcggacgcggccgccggctccagggagaccccgctgaaccaggaatccgcccgcaagagcgagccgcctgccccggtgcgcagacagagctattccagcaccagcagaggtatctcagtaacgaagaagacacatacatctcaaattgaaattattccatgcaagatctgtggagacaaatcatcaggaatccattatggtgtcattacatgtgaaggctgcaagggctttttcaggagaagtcagcaaagcaatgccacctactcctgtcctcgtcagaagaactgtttgattgatcgaaccagtagaaaccgctgccaacactgtcgattacagaaatgccttgccgtagggatgtctcgagatgctgtaaaatttggccgaatgtcaaaaaagcagagagacagcttgtatgcagaagtacagaaacaccggatgcagcagcagcagcgcgaccaccagcagcagcctggagaggctgagccgctgacgcccacctacaacatctcggccaacgggctgacggaacttcacgacgacctcagtaactacattgacgggcacacccctgaggggagtaaggcagactccgccgtcagcagcttctacctggacatacagccttccccagaccagtcaggtcttgatatcaatggaatcaaaccagaaccaatatgtgactacacaccagcatcaggcttctttccctactgttcgttcaccaacggcgagacttccccaactgtgtccatggcagaattagaacaccttgcacagaatatatctaaatcgcatctggaaacctgccaatacttgagagaagagctccagcagataacgtggcagacctttttacaggaagaaattgagaactatcaaaacaagcagcgggaggtgatgtggcaattgtgtgccatcaaaattacagaagctatacagtatgtggtggagtttgccaaacgcattgatggatttatggaactgtgtcaaaatgatcaaattgtgcttctaaaagcaggttctctagaggtggtgtttatcagaatgtgccgtgcctttgactctcagaacaacaccgtgtactttgatgggaagtatgccagccccgacgtcttcaaatccttaggttgtgaagactttattagctttgtgtttgaatttggaaagagtttatgttctatgcacctgactgaagatgaaattgcattattttctgcatttgtactgatgtcagcagatcgctcatggctgcaagaaaaggtaaaaattgaaaaactgcaacagaaaattcagctagctcttcaacacgtcctacagaagaatcaccgagaagatggaatactaacaaagttaatatgcaaggtgtctaccttaagagccttatgtggacgacatacagaaaagctaatggcatttaaagcaatatacccagacattgtgcgacttcattttcctccattatacaaggagttgttcacttcagaatttgagccagcaatgcaaattgatgggtaa

SEQ ID NO: 13 - DNA, 1380 bp, Human
atgcgagcacaaattgaagtgataccatgcaaaatttgtggcgataagtcctctgggatccactacggagtcatcacatgtgaaggctgcaagggattctttaggaggagccagcagaacaatgcttcttattcctgcccaaggcagagaaactgtttaattgacagaacgaacagaaaccgttgccaacactgccgactgcagaagtgtcttgccctaggaatgtcaagagatgctgtgaagtttgggaggatgtccaagaagcaaagggacagcctgtatgctgaggtgcagaagcaccagcagcggctgcaggaacagcggcagcagcagagtggggaggcagaagcccttgccagggtgtacagcagcagcattagcaacggcctgagcaacctgaacaacgagaccagcggcacttatgccaacgggcacgtcattgacctgcccaagtctgagggttattacaacgtcgattccggtcagccgtcccctgatcagtcaggacttgacatgactggaatcaaacagataaagcaagaacctatctatgacctcacatccgtacccaacttgtttacctatagctctttcaacaatgggcagttagcaccagggataaccatgactgaaatcgaccgaattgcacagaacatcattaagtcccatttggagacatgtcaatacaccatggaagagctgcaccagctggcgtggcagacccacacctatgaagaaattaaagcatatcaaagcaagtccagggaagcactgtggcaacaatgtgccatccagatcactcacgccatccaatacgtggtggagtttgcaaagcggataacaggcttcatggagctctgtcaaaatgatcaaattctacttctgaagtcaggttgcttggaagtggttttagtgagaatgtgccgtgccttcaacccattaaacaacactgttctgtttgaaggaaaatatggaggaatgcaaatgttcaaagccttaggttctgatgacctagtgaatgaagcatttgactttgcaaagaatttgtgttccttgcagctgaccgaggaggagatcgctttgttctcatctgctgttctgatatctccagaccgagcctggcttatagaaccaaggaaagtccagaagcttcaggaaaaaatttattttgcacttcaacatgtgattcagaagaatcacctggatgatgagaccttggcaaagttaatagccaagataccaaccatcacggcagtttgcaacttgcacggggagaagctgcaggtatttaagcaatctcatccagagatagtgaatacactgtttcctccgttatacaaggagctctttaatcctgactgtgccaccggctgcaaatga

SEQ ID NO: 14 - DNA, 1557 bp, Human
atggacagggccccacagagacagcaccgagcctcacgggagctgctggctgcaaagaagacccacacctcacaaattgaagtgatcccttgcaaaatctgtggggacaagtcgtctgggatccactacggggttatcacctgtgaggggtgcaagggcttcttccgccggagccagcgctgtaacgcggcctactcctgcacccgtcagcagaactgccccatcgaccgcaccagccgaaaccgatgccagcactgccgcctgcagaaatgcctggcgctgggcatgtcccgagatgctgtcaagttcggccgcatgtccaagaagcagagggacagcctgcatgcagaagtgcagaaacagctgcagcagcggcaacagcagcaacaggaaccagtggtcaagacccctccagcaggggcccaaggagcagataccctcacctacaccttggggctcccagacgggcagctgcccctgggctcctcgcctgacctgcctgaggcttctgcctgtccccctggcctcctgaaagcctcaggctctgggccctcatattccaacaacttggccaaggcagggctcaatggggcctcatgccaccttgaatacagccctgagcggggcaaggctgagggcagagagagcttctatagcacaggcagccagctgacccctgaccgatgtggacttcgttttgaggaacacaggcatcctgggcttggggaactgggacagggcccagacagctacggcagccccagtttccgcagcacaccggaggcaccctatgcctccctgacagagatagagcacctggtgcagagcgtctgcaagtcctacagggagacatgccagctgcggctggaggacctgctgcggcagcgctccaacatcttctcccgggaggaagtgactggctaccagaggaagtccatgtgggagatgtgggaacggtgtgcccaccacctcaccgaggccattcagtacgtggtggagttcgccaagaggctctcaggctttatggagctctgccagaatgaccagattgtgcttctcaaagcaggagcaatggaagtggtgctggttaggatgtgccgggcctacaatgctgacaaccgcacggtcttttttgaaggcaaatacggtggcatggagctgttccgagccttgggctgcagcgagctcatcagctccatctttgacttctcccactccctaagtgccttgcacttttccgaggatgagattgccctctacacagcccttgttctcatcaatgcccatcggccagggctccaagagaaaaggaaagtagaacagctgcagtacaatctggagctggcctttcatcatcatctctgcaagactcatcgccaaagcatcctggcaaagctgccacccaaggggaagcttcggagcctgtgtagccagcatgtggaaaggctgcagatcttccagcacctccaccccatcgtggtccaagccgctttccctccactctacaaggagctcttcagcactgaaaccgagtcacctgtggggctgtccaagtga

SEQ ID NO: 15 - DNA, 2592 bp, Human
atggcaaggctgggaaactgcagcctgacttgggctgccctgatcatcctgctgctccccggaagtctggaggagtgcgggcacatcagtgtctcagcccccatcgtccacctgggggatcccatcacagcctcctgcatcatcaagcagaactgcagccatctggacccggagccacagattctgtggagactgggagcagagcttcagcccgggggcaggcagcagcgtctgtctgatgggacccaggaatctatcatcaccctgccccacctcaaccacactcaggcctttctctcctgctgcctgaactggggcaacagcctgcagatcctggaccaggttgagctgcgcgcaggctaccctccagccataccccacaacctctcctgcctcatgaacctcacaaccagcagcctcatctgccagtgggagccaggacctgagacccacctacccaccagcttcactctgaagagtttcaagagccggggcaactgtcagacccaaggggactccatcctggactgcgtgcccaaggacgggcagagccactgctgcatcccacgcaaacacctgctgttgtaccagaatatgggcatctgggtgcaggcagagaatgcgctggggaccagcatgtccccacaactgtgtcttgatcccatggatgttgtgaaactggagccccccatgctgcggaccatggaccccagccctgaagcggcccctccccaggcaggctgcctacagctgtgctgggagccatggcagccaggcctgcacataaatcagaagtgtgagctgcgccacaagccgcagcgtggagaagccagctgggcactggtgggccccctccccttggaggcccttcagtatgagctctgcgggctcctcccagccacggcctacaccctgcagatacgctgcatccgctggcccctgcctggccactggagcgactggagccccagcctggagctgagaactaccgaacgggcccccactgtcagactggacacatggtggcggcagaggcagctggaccccaggacagtgcagctgttctggaagccagtgcccctggaggaagacagcggacggatccaaggttatgtggtttcttggagaccctcaggccaggctggggccatcctgcccctctgcaacaccacagagctcagctgcaccttccacctgccttcagaagcccaggaggtggcccttgtggcctataactcagccgggacctctcgtcccactccggtggtcttctcagaaagcagaggcccagctctgaccagactccatgccatggcccgagaccctcacagcctctgggtaggctgggagccccccaatccatggcctcagggctatgtgattgagtggggcctgggcccccccagcgcgagcaatagcaacaagacctggaggatggaacagaatgggagagccacggggtttctgctgaaggagaacatcaggccctttcagctctatgagatcatcgtgactcccttgtaccaggacaccatgggaccctcccagcatgtctatgcctactctcaagaaatggctccctcccatgccccagagctgcatctaaagcacattggcaagacctgggcacagctggagtgggtgcctgagccccctgagctggggaagagcccccttacccactacaccatcttctggaccaacgctcagaaccagtccttctccgccatcctgaatgcctcctcccgtggctttgtcctccatggcctggagcccgccagtctgtatcacatccacctcatggctgccagccaggctggggccaccaacagtacagtcctcaccctgatgaccttgaccccagaggggtcggagctacacatcatcctgggcctgttcggcctcctgctgttgctcacctgcctctgtggaactgcctggctctgttgcagccccaacaggaagaatcccctctggccaagtgtcccagacccagctcacagcagcctgggctcctgggtgcccacaatcatggaggagctgcccggacccagacagggacagtggctggggcagacatctgaaatgagccgtgctctcaccccacatccttgtgtgcaggatgccttccagctgcccggccttggcacgccacccatcaccaagctcacagtgctggaggaggatgaaaagaagccggtgccctgggagtcccataacagctcagagacctgtggcctccccactctggtccagacctatgtgctccagggggacccaagagcagtttccacccagccccaatcccagtctggcaccagcgatcaggtcctttatgggcagctgctgggcagccccacaagcccagggccagggcactatctccgctgtgactccactcagcccctcttggcgggcctcacccccagccccaagtcctatgagaacctctggttccaggccagccccttggggaccctggtaaccccagccccaagccaggaggacgactgtgtctttgggccactgctcaacttccccctcctgcaggggatccgggtccatgggatggaggcgctggggagcttctag

SEQ ID NO: 16 - DNA, 933 bp, Human
atgggaatcctgtcattcttacctgtccttgccactgagagtgactgggctgactgcaagtccccccagccttggggtcatatgcttctgtggacagctgtgctattcctggctcctgttgctgggacacctgcagctcccccaaaggctgtgctgaaactcgagccccagtggatcaacgtgctccaggaggactctgtgactctgacatgccgggggactcacagccctgagagcgactccattcagtggttccacaatgggaatctcattcccacccacacgcagcccagctacaggttcaaggccaacaacaatgacagcggggagtacacgtgccagactggccagaccagcctcagcgaccctgtgcatctgactgtgctttctgagtggctggtgctccagacccctcacctggagttccaggagggagaaaccatcgtgctgaggtgccacagctggaaggacaagcctctggtcaaggtcacattcttccagaatggaaaatccaagaaattttcccgttcggatcccaacttctccatcccacaagcaaaccacagtcacagtggtgattaccactgcacaggaaacataggctacacgctgtactcatccaagcctgtgaccatcactgtccaagctcccagctcttcaccgatggggatcattgtggctgtggtcactgggattgctgtagcggccattgttgctgctgtagtggccttgatctactgcaggaaaaagcggatttcagctctcccaggataccctgagtgcagggaaatgggagagaccctccctgagaaaccagccaatcccactaatcctgatgaggctgacaaagttggggctgagaacacaatcacctattcacttctcatgcacccggatgctctggaagagcctgatgaccagaaccgtatttag

SEQ ID NO: 17 - DNA, 894 bp, Human
atgacaacacccagaaattcagtaaatgggactttcccggcagagccaatgaaaggccctattgctatgcaatctggtccaaaaccactcttcaggaggatgtcttcactggtgggccccacgcaaagcttcttcatgagggaatctaagactttgggggctgtccagattatgaatgggctcttccacattgccctggggggtcttctgatgatcccagcagggatctatgcacccatctgtgtgactgtgtggtaccctctctggggaggcattatgtatattatttccggatcactcctggcagcaacggagaaaaactccaggaagtgtttggtcaaaggaaaaatgataatgaattcattgagcctctttgctgccatttctggaatgattctttcaatcatggacatacttaatattaaaatttcccattttttaaaaatggagagtctgaattttattagagctcacacaccatatattaacatatacaactgtgaaccagctaatccctctgagaaaaactccccatctacccaatactgttacagcatacaatctctgttcttgggcattttgtcagtgatgctgatctttgccttcttccaggaacttgtaatagctggcatcgttgagaatgaatggaaaagaacgtgctccagacccaaatctaacatagttctcctgtcagcagaagaaaaaaaagaacagactattgaaataaaagaagaagtggttgggctaactgaaacatcttcccaaccaaagaatgaagaagacattgaaattattccaatccaagaagaggaagaagaagaaacagagacgaactttccagaacctccccaagatcaggaatcctcaccaatagaaaatgacagctctccttaa

SEQ ID NO: 18 - DNA, 702 bp, Human
atgtggcagctgctcctcccaactgctctgctacttctagtttcagctggcatgcggactgaagatctcccaaaggctgtggtgttcctggagcctcaatggtacagcgtgcttgagaaggacagtgtgactctgaagtgccagggagcctactcccctgaggacaattccacacagtggtttcacaatgagaacctcatctcaagccaggcctcgagctacttcattgacgctgccacagtcaacgacagtggagagtacaggtgccagacaaacctctccaccctcagtgacccggtgcagctagaagtccatatcggctggctgttgctccaggcccctcggtgggtgttcaaggaggaagaccctattcacctgaggtgtcacagctggaagaacactgctctgcataaggtcacatatttacagaatggcaaagacaggaagtattttcatcataattctgacttccacattccaaaagccacactcaaagatagcggctcctacttctgcagggggcttgttgggagtaaaaatgtgtcttcagagactgtgaacatcaccatcactcaaggtttggcagtgtcaaccatctcatcattctctccacctgggtaccaagtctctttctgcttggtgatggtactcctttttgcagtggacacaggactatatttctctgtgaagacaaacatttga

SEQ ID NO: 19 - DNA, 2298 bp, Human
atgagtggggaccacctccacaacgattcccagatcgaagcggatttccgattgaatgattctcataaacacaaagataaacacaaagatcgagaacaccggcacaaagaacacaagaaggagaaggaccgggaaaagtccaagcatagcaacagtgaacataaagattctgaaaagaaacacaaagagaaggagaagaccaaacacaaagatggaagctcagaaaagcataaagacaaacataaagacagagacaaggaaaaacgaaaagaggaaaaggttcgagcctctggggatgcaaaaataaagaaggagaaggaaaatggcttctctagtccaccacaaattaaagatgaacctgaagatgatggctattttgttcctcctaaagaggatataaagccattaaagagacctcgagatgaggatgatgctgattataaacctaagaaaattaaaacagaagataccaagaaggagaagaaaagaaaactagaagaagaagaggatggtaaattgaaaaaacccaagaataaagataaagataaaaaagttcctgagccagataacaagaaaaagaagccgaagaaagaagaggaacagaagtggaaatggtgggaagaagagcgctatcctgaaggcatcaagtggaaattcctagaacataaaggtccagtatttgccccaccatatgagcctcttccagagaatgtcaagttttattatgatggtaaagtcatgaagctgagccccaaagcagaggaagtagctacgttctttgcaaaaatgctcgaccatgaatatactaccaaggaaatatttaggaaaaatttctttaaagactggagaaaggaaatgactaatgaagagaagaatattatcaccaacctaagcaaatgtgattttacccagatgagccagtatttcaaagcccagacggaagctcggaaacagatgagcaaggaagagaaactgaaaatcaaagaggagaatgaaaaattactgaaagaatatggattctgtattatggataaccacaaagagaggattgctaacttcaagatagagcctcctggacttttccgtggccgcggcaaccaccccaagatgggcatgctgaagagacgaatcatgcccgaggatataatcatcaactgtagcaaagatgccaaggttccttctcctcctccaggacataagtggaaagaagtccggcatgataacaaggttacttggctggtttcctggacagagaacatccaaggttccattaaatacatcatgcttaaccctagttcacgaatcaagggtgagaaggactggcagaaatacgagactgctcggcggctgaaaaaatgtgtggacaagatccggaaccagtatcgagaagactggaagtccaaagagatgaaagtccggcagagagctgtagccctgtacttcatcgacaagcttgctctgagagcaggcaatgaaaaggaggaaggagaaacagcggacactgtgggctgctgctcacttcgtgtggagcacatcaatctacacccagagttggatggtcaggaatatgtggtagagtttgacttcctcgggaaggactccatcagatactataacaaggtccctgttgagaaacgagtttttaagaacctacaactatttatggagaacaagcagcccgaggatgatctttttgatagactcaatactggtattctgaataagcatcttcaggatctcatggagggcttgacagccaaggtattccgtacatacaatgcctccatcacgctacagcagcagctaaaagaactgacagccccggatgagaacatcccagcgaagatcctttcttataaccgtgccaatcgagctgttgcaattctttgtaaccatcagagggcaccaccaaaaacttttgagaagtctatgatgaacttgcaaactaagattgatgccaagaaggaacagctagcagatgcccggagagacctgaaaagtgctaaggctgatgccaaggtcatgaaggatgcaaagacgaagaaggtagtagagtcaaagaagaaggctgttcagagactggaggaacagttgatgaagctggaagttcaagccacagaccgagaggaaaataaacagattgccctgggaacctccaaactcaattatctggaccctaggatcacagtggcttggtgcaagaagtggggtgtcccaattgagaagatttacaacaaaacccagcgggagaagtttgcctgggccattgacatggctgatgaagactatgagttttag